European Patent Specification EP 3 497 239 B1, published May 27, 2026. Title: ANALYSIS OF METHYLATION STATUS AND COPY NUMBER. Applicant: Ramot at Tel-Aviv University Ltd. Rheinisch-Westfalische Technische Hochschule (RWTH) Aachen EBENSTEIN, Yuval WEINHOLD, Elmar GRUNWALD, Assaf GABRIELI, Tslil. The sequence listing filed with the application follows.

SEQUENCE LISTING (1 sequence)

SEQ ID NO: 1 - DNA, 3220 bp, Homo sapiens
  misc_feature: D4Z4 repeat nucleic acid sequence
cccgggccagagctctcctgcctctccaccagcccaccccgccgcctgaccgccccctccccaccccccaccccccacccccggaaaacgcgtcgtcccctgggctgggtggagacccccgtcccgcgaaacaccgggccccgcgcagcgtccgggcctgacaccgctccgccggctcgcctcctcctgtcgcccccgggccaccgtcgcccgcccgcccgggcccctgcgggcccctgcagccgcccagctgccagcacgggcggctggcggcggaacgcagaccccaggcccggcgcacaccggggacgctgagcgttccaggcgggagggaaggcgggcagagatggagagaggaacgggagagactagaggggcggaagggacgttaggagggaggcagggaggcagggaggcagggaggaacggagggagagacagagcgacgcagggactgggggcggggccgagggagccggggacggacggggggaggaaggcagggaggaaaagcggtcctcggcctccgggagtagcgggaccgcccgcctccgggaaaacggtcagcgtccggcgcgggctgagggctgggcccacagccgccgcgccggccggcggggcaccacccattcgccccggttccggggcccagggagtgggcggtttcctccgggacaaaagaccgggactcgggttgccgtcgggtcttcacccgcgcggttcacagaccgcacatccccaggctgagccctgcaacgcggcgcgaggcccacagacccggccacggaggagccacacgcaggacgacggaggcgtgattttggtttccgagtggctttgccctcccgaaggcggcctgttgctcacgtctctccggcccccgaaaggctggccatgccgactgtttgctcccggagctctgcggcacccggaaacatgcagggaagggtgcaagcccggcatggtgccttcgctctccttgccaggttccaaacccgccacactgcagactcccccacgttgccgcacgcgggaatccatcgtcaggccatcacgccggggaggcatctcctctctggggtctcgctctggtcttctacgtggaaatgaacgagagccacacgcctgcgtgtgcgagaccgtcccggcaacggcgacgcccacaggcattgcctccttcacggagagagggcctggcacactcaagactcccacggaggttcagttccacactcccctccaccctcccaggctggtttctccctgctgccgacgcgtgggagcccagagagcggcttcccgttcccgcgggatccctggagaggtccggagagccggcccccgaaacgcgcccccctcccccctcccccctctcccccttcctcttcgtctctccggccccaccaccaccaccgccaccacgcctcccccaccaccccccccccccaccaccaccaccaccaccaccccgccggccggccccaggcctcgacgccctgggtcccttccggggtggggcgggctgtcccaggggggctcaccgccattcatgaaggggtggagcctgcctgcctgtgggcctttacaagggcggctggctggctggctggctgtccgggcaggcctcctggctgcacctgccgcagtgcacagtccggctgaggtgcacgggagcccgccggcctctctctgcccgcgtccgtccgtgaaattccggccggggctcaccgcgatggccctcccgacaccctcggacagcaccctccccgcggaagcccggggacgaggacggccacggagactcgtttggaccccgagccaaagcgaggccctgcgagcctgctttgagcggaacccgtacccgggcatcgccaccagagaacggctggcccaggccatcggcattccggagcccagggtccagatttggtttcagaatgagaggtcacgccagctgaggcagcaccggcgggaatctcggccctggcccgggagacgcggcccgccagaaggccggcgaaagcggaccgccgtcaccggatcccagaccgccctgctcctccgagcctttgagaaggatcgctttccaggcatcgccgcccgggaggagctggccagagagacgggcctcccggagtccaggattcagatctggtttcagaatcgaagggccaggcacccgggacagggtggcagggcgcccgcgcaggcaggcggcctgtgcagcgcggcccccggcgggggtcaccctgctccctcgtgggtcgccttcgcccacaccggcgcgtggggaacggggcttcccgcaccccacgtgccctgcgcgcctggggctctcccacagggggctttcgtgagccaggcagcgagggccgcccccgcgctgcagcccagccaggccgcgccggcagagggggtctcccaacctgccccggcgcgcggggatttcgcctacgccgccccggctcctccggagccggggcgctctcccaccctcaggctcctcggtggcctccgcacccgggcaaaagccgggaggaccgggacccgcagcgcgacggcctgccgggcccctgcgcggtggcacagcctgggcccgctcaagcggggccgcaggccaaggggtgcttgcgccacccacgtcccaggggagtccgtggtggggctggggccggggtccccaggtcgccggggcggcgtgggaaccccaagccggggcagctccacctccccagcccgcgcccccgggacgcctccgcctccgcgcggcaggggcagatgcaaggcatcccggcgccctcccaggcgctccaggagccggcgccctggtctgcactcccctgcggcctgctgctggatgagctcctggcgagcccggagtttctgcagcaggcgcaacctctcctagaaacggaggccccgggggagctggaggcctcggaagaggcgcctcgctggaagcacccctcagcgaggaagaataccgggctctgctggaggagctttaggacgcggggttgggacggggtcgggtggttcggggcagggcggtggcctctctttcgcggggaacacctggctggctacggaggggcgtgtctccgccccgccccctccaccgggctgaccggcctgggattcctgccttctaggtccaggcccggtgagagactccacaccgcggagaactgccattctttcctgggcatcccggggatcc